European Patent Specification EP 3 870 211 B1, published January 8, 2025. Title: Glucagon Like Peptide 1 (GLP1)-Growth Differentiation Factor 15 (GDF15) Fusion Proteins and Uses Thereof. Applicant: Janssen Pharmaceutica NV. The sequence listing filed with the application follows.

SEQUENCE LISTING (84 sequences)

SEQ ID NO: 1 - protein, 30 aa, Artificial Sequence
  (A8S, A30E) GLP-1(7-36)
HSEGTFTSDVSSYLEGQAAKEFIEWLVKGR

SEQ ID NO: 2 - protein, 30 aa, Artificial Sequence
  (A8G, G22E, R36G) GLP1(7-36)
HGEGTFTSDVSSYLEEQAAKEFIAWLVKGG

SEQ ID NO: 3 - protein, 39 aa, Artificial Sequence
  Exendin 4 (1-39)
HGEGTFTSDLSKQMEEEAVRLFIEWLKNGGPSSGAPPPS

SEQ ID NO: 4 - protein, 28 aa, Artificial Sequence
  Exendin 4 (1-28)
HGEGTFTSDLSKQMEEEAVRLFIEWLKN

SEQ ID NO: 5 - protein, 10 aa, Artificial Sequence
  First linker peptide 1-1
APAPAPAPAP

SEQ ID NO: 6 - protein, 20 aa, Artificial Sequence
  First linker peptide 1-2
APAPAPAPAPAPAPAPAPAP

SEQ ID NO: 7 - protein, 30 aa, Artificial Sequence
  First linker peptide 1-3
APAPAPAPAPAPAPAPAPAPAPAPAPAPAP

SEQ ID NO: 8 - protein, 40 aa, Artificial Sequence
  First linker peptide 1-4
APAPAPAPAPAPAPAPAPAPAPAPAPAPAPAPAPAPAPAP

SEQ ID NO: 9 - protein, 50 aa, Artificial Sequence
  First linker peptide 1-5
APAPAPAPAPAPAPAPAPAPAPAPAPAPAPAPAPAPAPAPAPAPAPAPAP

SEQ ID NO: 10 - protein, 24 aa, Artificial Sequence
  First linker peptide 1-6
ASAPAPAPAPAPAPAPAPAPAPGS

SEQ ID NO: 11 - protein, 14 aa, Artificial Sequence
  First linker peptide 1-7
ASAPAPAPAPAPGS

SEQ ID NO: 12 - protein, 12 aa, Artificial Sequence
  First linker peptide 1-8
ASGGGGSGGGGS

SEQ ID NO: 13 - protein, 42 aa, Artificial Sequence
  First linker peptide 1-9
ASGGGGSGGGGSGGGGSGGGGSGGGGSGGGGSGGGGSGGGGS

SEQ ID NO: 14 - protein, 12 aa, Artificial Sequence
  First linker peptide 1-10
GAGGGGAGGGGA

SEQ ID NO: 15 - protein, 42 aa, Artificial Sequence
  First linker peptide 1-11
GAGGGGAGGGGAGGGGAGGGGAGGGGAGGGGAGGGGAGGGGA

SEQ ID NO: 16 - protein, 15 aa, Artificial Sequence
  First linker peptide 1-12
GGGGAGGGGAGGGGA

SEQ ID NO: 17 - protein, 20 aa, Artificial Sequence
  First linker peptide 1-13
GGGGAGGGGAGGGGAGGGGA

SEQ ID NO: 18 - protein, 25 aa, Artificial Sequence
  First linker peptide 1-14
GGGGAGGGGAGGGGAGGGGAGGGGA

SEQ ID NO: 19 - protein, 30 aa, Artificial Sequence
  First linker peptide 1-15
GGGGAGGGGAGGGGAGGGGAGGGGAGGGGA

SEQ ID NO: 20 - protein, 40 aa, Artificial Sequence
  First linker peptide 1-16
GGGGAGGGGAGGGGAGGGGAGGGGAGGGGAGGGGAGGGGA

SEQ ID NO: 21 - protein, 20 aa, Artificial Sequence
  First linker peptide 1-17
GGGGGGGGGGGGGGGGGGGG

SEQ ID NO: 22 - protein, 25 aa, Artificial Sequence
  First linker peptide 1-18
GGGGGGGGGGGGGGGGGGGGGGGGG

SEQ ID NO: 23 - protein, 15 aa, Artificial Sequence
  First linker peptide 1-19
GGGGSGGGGSGGGGS

SEQ ID NO: 24 - protein, 25 aa, Artificial Sequence
  First linker peptide 1-20
GGGGSGGGGSGGGGSGGGGSGGGGS

SEQ ID NO: 25 - protein, 30 aa, Artificial Sequence
  First linker peptide 1-21
GGGGSGGGGSGGGGSGGGGSGGGGSGGGGS

SEQ ID NO: 26 - protein, 585 aa, Artificial Sequence
  HSA(C34S)
DAHKSEVAHRFKDLGEENFKALVLIAFAQYLQQSPFEDHVKLVNEVTEFAKTCVADESAENCDKSLHTLFGDKLCTVATLRETYGEMADCCAKQEPERNECFLQHKDDNPNLPRLVRPEVDVMCTAFHDNEETFLKKYLYEIARRHPYFYAPELLFFAKRYKAAFTECCQAADKAACLLPKLDELRDEGKASSAKQRLKCASLQKFGERAFKAWAVARLSQRFPKAEFAEVSKLVTDLTKVHTECCHGDLLECADDRADLAKYICENQDSISSKLKECCEKPLLEKSHCIAEVENDEMPADLPSLAADFVESKDVCKNYAEAKDVFLGMFLYEYARRHPDYSVVLLLRLAKTYETTLEKCCAAADPHECYAKVFDEFKPLVEEPQNLIKQNCELFEQLGEYKFQNALLVRYTKKVPQVSTPTLVEVSRNLGKVGSKCCKHPEAKRMPCAEDYLSVVLNQLCVLHEKTPVSDRVTKCCTESLVNRRPCFSALEVDETYVPKEFNAETFTFHADICTLSEKERQIKKQTALVELVKHKPKATKEQLKAVMDDFAAFVEKCCKADDKETCFAEEGKKLVAASQAALGL

SEQ ID NO: 27 - protein, 585 aa, Artificial Sequence
  GSA(C34S)
DAHKSEVAHRFKDLGEETFKALVLVAFAQYLQQSPFEDHVKLVNEVTEFAKTCVADESAENCDKSLHTLFGDKLCTVATLRETYGEMADCCAKQEPERNECFLQHKDDNPNLPRLVRPEVDVMCTAFHDNEETFLKKYLYEIARRHPYFYAPELLFFAARYKAAFTECCQAADKAACLLPKLDELRDEGKASSAKQRLKCASLQKFGERAFKAWAVARLSQRFPKAEFAEVSKLVTDLTKVHTECCHGDLLECADDRADLAKYICENQDSISSKLKECCEKPLLEKSHCLAEVENDEMPADLPSLAADFVESKDVCKNYAEAKDVFLGMFLYEYARRHPDYSVVLLLRLAKTYETTLEKCCAAADPHECYAKVFDEFKPLVEEPQNLIKQNCELFEQLGEYKFQNALLVRYTKKVPQVSTPTLVEVSRNLGKVGSKCCKHPEAKRMPCAEDYLSVVLNQLCVLHEKTPVSDRVTKCCTESLVNRRPCFSALEVDETYVPKEFNAETFTFHADICTLSEKERQIKKQTALAELVKHKPKATKEQLKTVMDDFAAFVEKCCKADDKETCFAEEGKKLVAASQAALGL

SEQ ID NO: 28 - protein, 20 aa, Artificial Sequence
  Second linker peptide 2-1
APAPAPAPAPAPAPAPAPAP

SEQ ID NO: 29 - protein, 42 aa, Artificial Sequence; identical to SEQ ID NO: 15
  Second linker peptide 2-2

SEQ ID NO: 30 - protein, 42 aa, Artificial Sequence
  Second linker peptide 2-3
GSGGGGSGGGGSGGGGSGGGGSGGGGSGGGGSGGGGSGGGGS

SEQ ID NO: 31 - protein, 108 aa, Artificial Sequence
  GDF15 variant 1
DHCPLGPGRCCRLHTVRASLEDLGWADWVLSPREVQVTMCIGACPSQFRAANMHAQIKTSLHRLKPDTVPAPCCVPASYNPMVLIQKTDTGVSLQTYDDLLAKDCHCI

SEQ ID NO: 32 - protein, 112 aa, Artificial Sequence
  GDF15 WT mature
ARNGDHCPLGPGRCCRLHTVRASLEDLGWADWVLSPREVQVTMCIGACPSQFRAANMHAQIKTSLHRLKPDTVPAPCCVPASYNPMVLIQKTDTGVSLQTYDDLLAKDCHCI

SEQ ID NO: 33 - protein, 768 aa, Artificial Sequence
  GLP1-GDF15 Fusion Protein 1
HGEGTFTSDVSSYLEEQAAKEFIAWLVKGGGGGGAGGGGAGGGGAGGGGAGGGGADAHKSEVAHRFKDLGEENFKALVLIAFAQYLQQSPFEDHVKLVNEVTEFAKTCVADESAENCDKSLHTLFGDKLCTVATLRETYGEMADCCAKQEPERNECFLQHKDDNPNLPRLVRPEVDVMCTAFHDNEETFLKKYLYEIARRHPYFYAPELLFFAKRYKAAFTECCQAADKAACLLPKLDELRDEGKASSAKQRLKCASLQKFGERAFKAWAVARLSQRFPKAEFAEVSKLVTDLTKVHTECCHGDLLECADDRADLAKYICENQDSISSKLKECCEKPLLEKSHCIAEVENDEMPADLPSLAADFVESKDVCKNYAEAKDVFLGMFLYEYARRHPDYSVVLLLRLAKTYETTLEKCCAAADPHECYAKVFDEFKPLVEEPQNLIKQNCELFEQLGEYKFQNALLVRYTKKVPQVSTPTLVEVSRNLGKVGSKCCKHPEAKRMPCAEDYLSVVLNQLCVLHEKTPVSDRVTKCCTESLVNRRPCFSALEVDETYVPKEFNAETFTFHADICTLSEKERQIKKQTALVELVKHKPKATKEQLKAVMDDFAAFVEKCCKADDKETCFAEEGKKLVAASQAALGLAPAPAPAPAPAPAPAPAPAPDHCPLGPGRCCRLHTVRASLEDLGWADWVLSPREVQVTMCIGACPSQFRAANMHAQIKTSLHRLKPDTVPAPCCVPASYNPMVLIQKTDTGVSLQTYDDLLAKDCHCI

SEQ ID NO: 34 - protein, 758 aa, Artificial Sequence
  GLP1-GDF15 Fusion Protein 2
HGEGTFTSDVSSYLEEQAAKEFIAWLVKGGGGGGAGGGGAGGGGADAHKSEVAHRFKDLGEENFKALVLIAFAQYLQQSPFEDHVKLVNEVTEFAKTCVADESAENCDKSLHTLFGDKLCTVATLRETYGEMADCCAKQEPERNECFLQHKDDNPNLPRLVRPEVDVMCTAFHDNEETFLKKYLYEIARRHPYFYAPELLFFAKRYKAAFTECCQAADKAACLLPKLDELRDEGKASSAKQRLKCASLQKFGERAFKAWAVARLSQRFPKAEFAEVSKLVTDLTKVHTECCHGDLLECADDRADLAKYICENQDSISSKLKECCEKPLLEKSHCIAEVENDEMPADLPSLAADFVESKDVCKNYAEAKDVFLGMFLYEYARRHPDYSVVLLLRLAKTYETTLEKCCAAADPHECYAKVFDEFKPLVEEPQNLIKQNCELFEQLGEYKFQNALLVRYTKKVPQVSTPTLVEVSRNLGKVGSKCCKHPEAKRMPCAEDYLSVVLNQLCVLHEKTPVSDRVTKCCTESLVNRRPCFSALEVDETYVPKEFNAETFTFHADICTLSEKERQIKKQTALVELVKHKPKATKEQLKAVMDDFAAFVEKCCKADDKETCFAEEGKKLVAASQAALGLAPAPAPAPAPAPAPAPAPAPDHCPLGPGRCCRLHTVRASLEDLGWADWVLSPREVQVTMCIGACPSQFRAANMHAQIKTSLHRLKPDTVPAPCCVPASYNPMVLIQKTDTGVSLQTYDDLLAKDCHCI

SEQ ID NO: 35 - protein, 793 aa, Artificial Sequence
  GLP1-GDF15 Fusion Protein 3
HGEGTFTSDVSSYLEEQAAKEFIAWLVKGGAPAPAPAPAPAPAPAPAPAPAPAPAPAPAPAPAPAPAPAPAPAPAPAPAPDAHKSEVAHRFKDLGEENFKALVLIAFAQYLQQSPFEDHVKLVNEVTEFAKTCVADESAENCDKSLHTLFGDKLCTVATLRETYGEMADCCAKQEPERNECFLQHKDDNPNLPRLVRPEVDVMCTAFHDNEETFLKKYLYEIARRHPYFYAPELLFFAKRYKAAFTECCQAADKAACLLPKLDELRDEGKASSAKQRLKCASLQKFGERAFKAWAVARLSQRFPKAEFAEVSKLVTDLTKVHTECCHGDLLECADDRADLAKYICENQDSISSKLKECCEKPLLEKSHCIAEVENDEMPADLPSLAADFVESKDVCKNYAEAKDVFLGMFLYEYARRHPDYSVVLLLRLAKTYETTLEKCCAAADPHECYAKVFDEFKPLVEEPQNLIKQNCELFEQLGEYKFQNALLVRYTKKVPQVSTPTLVEVSRNLGKVGSKCCKHPEAKRMPCAEDYLSVVLNQLCVLHEKTPVSDRVTKCCTESLVNRRPCFSALEVDETYVPKEFNAETFTFHADICTLSEKERQIKKQTALVELVKHKPKATKEQLKAVMDDFAAFVEKCCKADDKETCFAEEGKKLVAASQAALGLAPAPAPAPAPAPAPAPAPAPDHCPLGPGRCCRLHTVRASLEDLGWADWVLSPREVQVTMCIGACPSQFRAANMHAQIKTSLHRLKPDTVPAPCCVPASYNPMVLIQKTDTGVSLQTYDDLLAKDCHCI

SEQ ID NO: 36 - protein, 783 aa, Artificial Sequence
  GLP1-GDF15 Fusion Protein 4
HGEGTFTSDVSSYLEEQAAKEFIAWLVKGGAPAPAPAPAPAPAPAPAPAPAPAPAPAPAPAPAPAPAPAPDAHKSEVAHRFKDLGEENFKALVLIAFAQYLQQSPFEDHVKLVNEVTEFAKTCVADESAENCDKSLHTLFGDKLCTVATLRETYGEMADCCAKQEPERNECFLQHKDDNPNLPRLVRPEVDVMCTAFHDNEETFLKKYLYEIARRHPYFYAPELLFFAKRYKAAFTECCQAADKAACLLPKLDELRDEGKASSAKQRLKCASLQKFGERAFKAWAVARLSQRFPKAEFAEVSKLVTDLTKVHTECCHGDLLECADDRADLAKYICENQDSISSKLKECCEKPLLEKSHCIAEVENDEMPADLPSLAADFVESKDVCKNYAEAKDVFLGMFLYEYARRHPDYSVVLLLRLAKTYETTLEKCCAAADPHECYAKVFDEFKPLVEEPQNLIKQNCELFEQLGEYKFQNALLVRYTKKVPQVSTPTLVEVSRNLGKVGSKCCKHPEAKRMPCAEDYLSVVLNQLCVLHEKTPVSDRVTKCCTESLVNRRPCFSALEVDETYVPKEFNAETFTFHADICTLSEKERQIKKQTALVELVKHKPKATKEQLKAVMDDFAAFVEKCCKADDKETCFAEEGKKLVAASQAALGLAPAPAPAPAPAPAPAPAPAPDHCPLGPGRCCRLHTVRASLEDLGWADWVLSPREVQVTMCIGACPSQFRAANMHAQIKTSLHRLKPDTVPAPCCVPASYNPMVLIQKTDTGVSLQTYDDLLAKDCHCI

SEQ ID NO: 37 - protein, 773 aa, Artificial Sequence
  GLP1-GDF15 Fusion Protein 5
HGEGTFTSDVSSYLEEQAAKEFIAWLVKGGAPAPAPAPAPAPAPAPAPAPAPAPAPAPAPDAHKSEVAHRFKDLGEENFKALVLIAFAQYLQQSPFEDHVKLVNEVTEFAKTCVADESAENCDKSLHTLFGDKLCTVATLRETYGEMADCCAKQEPERNECFLQHKDDNPNLPRLVRPEVDVMCTAFHDNEETFLKKYLYEIARRHPYFYAPELLFFAKRYKAAFTECCQAADKAACLLPKLDELRDEGKASSAKQRLKCASLQKFGERAFKAWAVARLSQRFPKAEFAEVSKLVTDLTKVHTECCHGDLLECADDRADLAKYICENQDSISSKLKECCEKPLLEKSHCIAEVENDEMPADLPSLAADFVESKDVCKNYAEAKDVFLGMFLYEYARRHPDYSVVLLLRLAKTYETTLEKCCAAADPHECYAKVFDEFKPLVEEPQNLIKQNCELFEQLGEYKFQNALLVRYTKKVPQVSTPTLVEVSRNLGKVGSKCCKHPEAKRMPCAEDYLSVVLNQLCVLHEKTPVSDRVTKCCTESLVNRRPCFSALEVDETYVPKEFNAETFTFHADICTLSEKERQIKKQTALVELVKHKPKATKEQLKAVMDDFAAFVEKCCKADDKETCFAEEGKKLVAASQAALGLAPAPAPAPAPAPAPAPAPAPDHCPLGPGRCCRLHTVRASLEDLGWADWVLSPREVQVTMCIGACPSQFRAANMHAQIKTSLHRLKPDTVPAPCCVPASYNPMVLIQKTDTGVSLQTYDDLLAKDCHCI

SEQ ID NO: 38 - protein, 783 aa, Artificial Sequence
  GLP1-GDF15 Fusion Protein 6
HGEGTFTSDVSSYLEEQAAKEFIAWLVKGGGGGGAGGGGAGGGGAGGGGAGGGGAGGGGAGGGGAGGGGADAHKSEVAHRFKDLGEENFKALVLIAFAQYLQQSPFEDHVKLVNEVTEFAKTCVADESAENCDKSLHTLFGDKLCTVATLRETYGEMADCCAKQEPERNECFLQHKDDNPNLPRLVRPEVDVMCTAFHDNEETFLKKYLYEIARRHPYFYAPELLFFAKRYKAAFTECCQAADKAACLLPKLDELRDEGKASSAKQRLKCASLQKFGERAFKAWAVARLSQRFPKAEFAEVSKLVTDLTKVHTECCHGDLLECADDRADLAKYICENQDSISSKLKECCEKPLLEKSHCIAEVENDEMPADLPSLAADFVESKDVCKNYAEAKDVFLGMFLYEYARRHPDYSVVLLLRLAKTYETTLEKCCAAADPHECYAKVFDEFKPLVEEPQNLIKQNCELFEQLGEYKFQNALLVRYTKKVPQVSTPTLVEVSRNLGKVGSKCCKHPEAKRMPCAEDYLSVVLNQLCVLHEKTPVSDRVTKCCTESLVNRRPCFSALEVDETYVPKEFNAETFTFHADICTLSEKERQIKKQTALVELVKHKPKATKEQLKAVMDDFAAFVEKCCKADDKETCFAEEGKKLVAASQAALGLAPAPAPAPAPAPAPAPAPAPDHCPLGPGRCCRLHTVRASLEDLGWADWVLSPREVQVTMCIGACPSQFRAANMHAQIKTSLHRLKPDTVPAPCCVPASYNPMVLIQKTDTGVSLQTYDDLLAKDCHCI

SEQ ID NO: 39 - protein, 802 aa, Artificial Sequence
  GLP1-GDF15 Fusion Protein 7
HGEGTFTSDLSKQMEEEAVRLFIEWLKNGGPSSGAPPPSAPAPAPAPAPAPAPAPAPAPAPAPAPAPAPAPAPAPAPAPAPAPAPAPAPDAHKSEVAHRFKDLGEENFKALVLIAFAQYLQQSPFEDHVKLVNEVTEFAKTCVADESAENCDKSLHTLFGDKLCTVATLRETYGEMADCCAKQEPERNECFLQHKDDNPNLPRLVRPEVDVMCTAFHDNEETFLKKYLYEIARRHPYFYAPELLFFAKRYKAAFTECCQAADKAACLLPKLDELRDEGKASSAKQRLKCASLQKFGERAFKAWAVARLSQRFPKAEFAEVSKLVTDLTKVHTECCHGDLLECADDRADLAKYICENQDSISSKLKECCEKPLLEKSHCIAEVENDEMPADLPSLAADFVESKDVCKNYAEAKDVFLGMFLYEYARRHPDYSVVLLLRLAKTYETTLEKCCAAADPHECYAKVFDEFKPLVEEPQNLIKQNCELFEQLGEYKFQNALLVRYTKKVPQVSTPTLVEVSRNLGKVGSKCCKHPEAKRMPCAEDYLSVVLNQLCVLHEKTPVSDRVTKCCTESLVNRRPCFSALEVDETYVPKEFNAETFTFHADICTLSEKERQIKKQTALVELVKHKPKATKEQLKAVMDDFAAFVEKCCKADDKETCFAEEGKKLVAASQAALGLAPAPAPAPAPAPAPAPAPAPDHCPLGPGRCCRLHTVRASLEDLGWADWVLSPREVQVTMCIGACPSQFRAANMHAQIKTSLHRLKPDTVPAPCCVPASYNPMVLIQKTDTGVSLQTYDDLLAKDCHCI

SEQ ID NO: 40 - protein, 782 aa, Artificial Sequence
  GLP1-GDF15 Fusion Protein 8
HGEGTFTSDLSKQMEEEAVRLFIEWLKNGGPSSGAPPPSAPAPAPAPAPAPAPAPAPAPAPAPAPAPAPDAHKSEVAHRFKDLGEENFKALVLIAFAQYLQQSPFEDHVKLVNEVTEFAKTCVADESAENCDKSLHTLFGDKLCTVATLRETYGEMADCCAKQEPERNECFLQHKDDNPNLPRLVRPEVDVMCTAFHDNEETFLKKYLYEIARRHPYFYAPELLFFAKRYKAAFTECCQAADKAACLLPKLDELRDEGKASSAKQRLKCASLQKFGERAFKAWAVARLSQRFPKAEFAEVSKLVTDLTKVHTECCHGDLLECADDRADLAKYICENQDSISSKLKECCEKPLLEKSHCIAEVENDEMPADLPSLAADFVESKDVCKNYAEAKDVFLGMFLYEYARRHPDYSVVLLLRLAKTYETTLEKCCAAADPHECYAKVFDEFKPLVEEPQNLIKQNCELFEQLGEYKFQNALLVRYTKKVPQVSTPTLVEVSRNLGKVGSKCCKHPEAKRMPCAEDYLSVVLNQLCVLHEKTPVSDRVTKCCTESLVNRRPCFSALEVDETYVPKEFNAETFTFHADICTLSEKERQIKKQTALVELVKHKPKATKEQLKAVMDDFAAFVEKCCKADDKETCFAEEGKKLVAASQAALGLAPAPAPAPAPAPAPAPAPAPDHCPLGPGRCCRLHTVRASLEDLGWADWVLSPREVQVTMCIGACPSQFRAANMHAQIKTSLHRLKPDTVPAPCCVPASYNPMVLIQKTDTGVSLQTYDDLLAKDCHCI

SEQ ID NO: 41 - protein, 772 aa, Artificial Sequence
  GLP1-GDF15 Fusion Protein 9
HGEGTFTSDLSKQMEEEAVRLFIEWLKNGGPSSGAPPPSAPAPAPAPAPAPAPAPAPAPDAHKSEVAHRFKDLGEENFKALVLIAFAQYLQQSPFEDHVKLVNEVTEFAKTCVADESAENCDKSLHTLFGDKLCTVATLRETYGEMADCCAKQEPERNECFLQHKDDNPNLPRLVRPEVDVMCTAFHDNEETFLKKYLYEIARRHPYFYAPELLFFAKRYKAAFTECCQAADKAACLLPKLDELRDEGKASSAKQRLKCASLQKFGERAFKAWAVARLSQRFPKAEFAEVSKLVTDLTKVHTECCHGDLLECADDRADLAKYICENQDSISSKLKECCEKPLLEKSHCIAEVENDEMPADLPSLAADFVESKDVCKNYAEAKDVFLGMFLYEYARRHPDYSVVLLLRLAKTYETTLEKCCAAADPHECYAKVFDEFKPLVEEPQNLIKQNCELFEQLGEYKFQNALLVRYTKKVPQVSTPTLVEVSRNLGKVGSKCCKHPEAKRMPCAEDYLSVVLNQLCVLHEKTPVSDRVTKCCTESLVNRRPCFSALEVDETYVPKEFNAETFTFHADICTLSEKERQIKKQTALVELVKHKPKATKEQLKAVMDDFAAFVEKCCKADDKETCFAEEGKKLVAASQAALGLAPAPAPAPAPAPAPAPAPAPDHCPLGPGRCCRLHTVRASLEDLGWADWVLSPREVQVTMCIGACPSQFRAANMHAQIKTSLHRLKPDTVPAPCCVPASYNPMVLIQKTDTGVSLQTYDDLLAKDCHCI

SEQ ID NO: 42 - protein, 792 aa, Artificial Sequence
  GLP1-GDF15 Fusion Protein 10
HGEGTFTSDLSKQMEEEAVRLFIEWLKNGGPSSGAPPPSGGGGAGGGGAGGGGAGGGGAGGGGAGGGGAGGGGAGGGGADAHKSEVAHRFKDLGEENFKALVLIAFAQYLQQSPFEDHVKLVNEVTEFAKTCVADESAENCDKSLHTLFGDKLCTVATLRETYGEMADCCAKQEPERNECFLQHKDDNPNLPRLVRPEVDVMCTAFHDNEETFLKKYLYEIARRHPYFYAPELLFFAKRYKAAFTECCQAADKAACLLPKLDELRDEGKASSAKQRLKCASLQKFGERAFKAWAVARLSQRFPKAEFAEVSKLVTDLTKVHTECCHGDLLECADDRADLAKYICENQDSISSKLKECCEKPLLEKSHCIAEVENDEMPADLPSLAADFVESKDVCKNYAEAKDVFLGMFLYEYARRHPDYSVVLLLRLAKTYETTLEKCCAAADPHECYAKVFDEFKPLVEEPQNLIKQNCELFEQLGEYKFQNALLVRYTKKVPQVSTPTLVEVSRNLGKVGSKCCKHPEAKRMPCAEDYLSVVLNQLCVLHEKTPVSDRVTKCCTESLVNRRPCFSALEVDETYVPKEFNAETFTFHADICTLSEKERQIKKQTALVELVKHKPKATKEQLKAVMDDFAAFVEKCCKADDKETCFAEEGKKLVAASQAALGLAPAPAPAPAPAPAPAPAPAPDHCPLGPGRCCRLHTVRASLEDLGWADWVLSPREVQVTMCIGACPSQFRAANMHAQIKTSLHRLKPDTVPAPCCVPASYNPMVLIQKTDTGVSLQTYDDLLAKDCHCI

SEQ ID NO: 43 - protein, 777 aa, Artificial Sequence
  GLP1-GDF15 Fusion Protein 11
HGEGTFTSDLSKQMEEEAVRLFIEWLKNGGPSSGAPPPSGGGGAGGGGAGGGGAGGGGAGGGGADAHKSEVAHRFKDLGEENFKALVLIAFAQYLQQSPFEDHVKLVNEVTEFAKTCVADESAENCDKSLHTLFGDKLCTVATLRETYGEMADCCAKQEPERNECFLQHKDDNPNLPRLVRPEVDVMCTAFHDNEETFLKKYLYEIARRHPYFYAPELLFFAKRYKAAFTECCQAADKAACLLPKLDELRDEGKASSAKQRLKCASLQKFGERAFKAWAVARLSQRFPKAEFAEVSKLVTDLTKVHTECCHGDLLECADDRADLAKYICENQDSISSKLKECCEKPLLEKSHCIAEVENDEMPADLPSLAADFVESKDVCKNYAEAKDVFLGMFLYEYARRHPDYSVVLLLRLAKTYETTLEKCCAAADPHECYAKVFDEFKPLVEEPQNLIKQNCELFEQLGEYKFQNALLVRYTKKVPQVSTPTLVEVSRNLGKVGSKCCKHPEAKRMPCAEDYLSVVLNQLCVLHEKTPVSDRVTKCCTESLVNRRPCFSALEVDETYVPKEFNAETFTFHADICTLSEKERQIKKQTALVELVKHKPKATKEQLKAVMDDFAAFVEKCCKADDKETCFAEEGKKLVAASQAALGLAPAPAPAPAPAPAPAPAPAPDHCPLGPGRCCRLHTVRASLEDLGWADWVLSPREVQVTMCIGACPSQFRAANMHAQIKTSLHRLKPDTVPAPCCVPASYNPMVLIQKTDTGVSLQTYDDLLAKDCHCI

SEQ ID NO: 44 - protein, 762 aa, Artificial Sequence
  GLP1-GDF15 Fusion Protein 12
HGEGTFTSDLSKQMEEEAVRLFIEWLKNGGPSSGAPPPSAPAPAPAPAPDAHKSEVAHRFKDLGEENFKALVLIAFAQYLQQSPFEDHVKLVNEVTEFAKTCVADESAENCDKSLHTLFGDKLCTVATLRETYGEMADCCAKQEPERNECFLQHKDDNPNLPRLVRPEVDVMCTAFHDNEETFLKKYLYEIARRHPYFYAPELLFFAKRYKAAFTECCQAADKAACLLPKLDELRDEGKASSAKQRLKCASLQKFGERAFKAWAVARLSQRFPKAEFAEVSKLVTDLTKVHTECCHGDLLECADDRADLAKYICENQDSISSKLKECCEKPLLEKSHCIAEVENDEMPADLPSLAADFVESKDVCKNYAEAKDVFLGMFLYEYARRHPDYSVVLLLRLAKTYETTLEKCCAAADPHECYAKVFDEFKPLVEEPQNLIKQNCELFEQLGEYKFQNALLVRYTKKVPQVSTPTLVEVSRNLGKVGSKCCKHPEAKRMPCAEDYLSVVLNQLCVLHEKTPVSDRVTKCCTESLVNRRPCFSALEVDETYVPKEFNAETFTFHADICTLSEKERQIKKQTALVELVKHKPKATKEQLKAVMDDFAAFVEKCCKADDKETCFAEEGKKLVAASQAALGLAPAPAPAPAPAPAPAPAPAPDHCPLGPGRCCRLHTVRASLEDLGWADWVLSPREVQVTMCIGACPSQFRAANMHAQIKTSLHRLKPDTVPAPCCVPASYNPMVLIQKTDTGVSLQTYDDLLAKDCHCI

SEQ ID NO: 45 - protein, 763 aa, Artificial Sequence
  GLP1-GDF15 Fusion Protein 13
HGEGTFTSDVSSYLEEQAAKEFIAWLVKGGAPAPAPAPAPAPAPAPAPAPDAHKSEVAHRFKDLGEENFKALVLIAFAQYLQQSPFEDHVKLVNEVTEFAKTCVADESAENCDKSLHTLFGDKLCTVATLRETYGEMADCCAKQEPERNECFLQHKDDNPNLPRLVRPEVDVMCTAFHDNEETFLKKYLYEIARRHPYFYAPELLFFAKRYKAAFTECCQAADKAACLLPKLDELRDEGKASSAKQRLKCASLQKFGERAFKAWAVARLSQRFPKAEFAEVSKLVTDLTKVHTECCHGDLLECADDRADLAKYICENQDSISSKLKECCEKPLLEKSHCIAEVENDEMPADLPSLAADFVESKDVCKNYAEAKDVFLGMFLYEYARRHPDYSVVLLLRLAKTYETTLEKCCAAADPHECYAKVFDEFKPLVEEPQNLIKQNCELFEQLGEYKFQNALLVRYTKKVPQVSTPTLVEVSRNLGKVGSKCCKHPEAKRMPCAEDYLSVVLNQLCVLHEKTPVSDRVTKCCTESLVNRRPCFSALEVDETYVPKEFNAETFTFHADICTLSEKERQIKKQTALVELVKHKPKATKEQLKAVMDDFAAFVEKCCKADDKETCFAEEGKKLVAASQAALGLAPAPAPAPAPAPAPAPAPAPDHCPLGPGRCCRLHTVRASLEDLGWADWVLSPREVQVTMCIGACPSQFRAANMHAQIKTSLHRLKPDTVPAPCCVPASYNPMVLIQKTDTGVSLQTYDDLLAKDCHCI

SEQ ID NO: 46 - protein, 784 aa, Artificial Sequence
  GLP1-GDF15 Fusion Protein 14
HGEGTFTSDLSKQMEEEAVRLFIEWLKNGGPSSGAPPPSAPAPAPAPAPDAHKSEVAHRFKDLGEENFKALVLIAFAQYLQQSPFEDHVKLVNEVTEFAKTCVADESAENCDKSLHTLFGDKLCTVATLRETYGEMADCCAKQEPERNECFLQHKDDNPNLPRLVRPEVDVMCTAFHDNEETFLKKYLYEIARRHPYFYAPELLFFAKRYKAAFTECCQAADKAACLLPKLDELRDEGKASSAKQRLKCASLQKFGERAFKAWAVARLSQRFPKAEFAEVSKLVTDLTKVHTECCHGDLLECADDRADLAKYICENQDSISSKLKECCEKPLLEKSHCIAEVENDEMPADLPSLAADFVESKDVCKNYAEAKDVFLGMFLYEYARRHPDYSVVLLLRLAKTYETTLEKCCAAADPHECYAKVFDEFKPLVEEPQNLIKQNCELFEQLGEYKFQNALLVRYTKKVPQVSTPTLVEVSRNLGKVGSKCCKHPEAKRMPCAEDYLSVVLNQLCVLHEKTPVSDRVTKCCTESLVNRRPCFSALEVDETYVPKEFNAETFTFHADICTLSEKERQIKKQTALVELVKHKPKATKEQLKAVMDDFAAFVEKCCKADDKETCFAEEGKKLVAASQAALGLGAGGGGAGGGGAGGGGAGGGGAGGGGAGGGGAGGGGAGGGGADHCPLGPGRCCRLHTVRASLEDLGWADWVLSPREVQVTMCIGACPSQFRAANMHAQIKTSLHRLKPDTVPAPCCVPASYNPMVLIQKTDTGVSLQTYDDLLAKDCHCI

SEQ ID NO: 47 - protein, 790 aa, Artificial Sequence
  GLP1-GDF15 Fusion Protein 15
HGEGTFTSDVSSYLEEQAAKEFIAWLVKGGGGGGGGGGGGGGGGGGGGGGGGGGGDAHKSEVAHRFKDLGEENFKALVLIAFAQYLQQSPFEDHVKLVNEVTEFAKTCVADESAENCDKSLHTLFGDKLCTVATLRETYGEMADCCAKQEPERNECFLQHKDDNPNLPRLVRPEVDVMCTAFHDNEETFLKKYLYEIARRHPYFYAPELLFFAKRYKAAFTECCQAADKAACLLPKLDELRDEGKASSAKQRLKCASLQKFGERAFKAWAVARLSQRFPKAEFAEVSKLVTDLTKVHTECCHGDLLECADDRADLAKYICENQDSISSKLKECCEKPLLEKSHCIAEVENDEMPADLPSLAADFVESKDVCKNYAEAKDVFLGMFLYEYARRHPDYSVVLLLRLAKTYETTLEKCCAAADPHECYAKVFDEFKPLVEEPQNLIKQNCELFEQLGEYKFQNALLVRYTKKVPQVSTPTLVEVSRNLGKVGSKCCKHPEAKRMPCAEDYLSVVLNQLCVLHEKTPVSDRVTKCCTESLVNRRPCFSALEVDETYVPKEFNAETFTFHADICTLSEKERQIKKQTALVELVKHKPKATKEQLKAVMDDFAAFVEKCCKADDKETCFAEEGKKLVAASQAALGLGAGGGGAGGGGAGGGGAGGGGAGGGGAGGGGAGGGGAGGGGADHCPLGPGRCCRLHTVRASLEDLGWADWVLSPREVQVTMCIGACPSQFRAANMHAQIKTSLHRLKPDTVPAPCCVPASYNPMVLIQKTDTGVSLQTYDDLLAKDCHCI

SEQ ID NO: 48 - protein, 785 aa, Artificial Sequence
  GLP1-GDF15 Fusion Protein 16
HGEGTFTSDVSSYLEEQAAKEFIAWLVKGGGGGGGGGGGGGGGGGGGGGGDAHKSEVAHRFKDLGEENFKALVLIAFAQYLQQSPFEDHVKLVNEVTEFAKTCVADESAENCDKSLHTLFGDKLCTVATLRETYGEMADCCAKQEPERNECFLQHKDDNPNLPRLVRPEVDVMCTAFHDNEETFLKKYLYEIARRHPYFYAPELLFFAKRYKAAFTECCQAADKAACLLPKLDELRDEGKASSAKQRLKCASLQKFGERAFKAWAVARLSQRFPKAEFAEVSKLVTDLTKVHTECCHGDLLECADDRADLAKYICENQDSISSKLKECCEKPLLEKSHCIAEVENDEMPADLPSLAADFVESKDVCKNYAEAKDVFLGMFLYEYARRHPDYSVVLLLRLAKTYETTLEKCCAAADPHECYAKVFDEFKPLVEEPQNLIKQNCELFEQLGEYKFQNALLVRYTKKVPQVSTPTLVEVSRNLGKVGSKCCKHPEAKRMPCAEDYLSVVLNQLCVLHEKTPVSDRVTKCCTESLVNRRPCFSALEVDETYVPKEFNAETFTFHADICTLSEKERQIKKQTALVELVKHKPKATKEQLKAVMDDFAAFVEKCCKADDKETCFAEEGKKLVAASQAALGLGAGGGGAGGGGAGGGGAGGGGAGGGGAGGGGAGGGGAGGGGADHCPLGPGRCCRLHTVRASLEDLGWADWVLSPREVQVTMCIGACPSQFRAANMHAQIKTSLHRLKPDTVPAPCCVPASYNPMVLIQKTDTGVSLQTYDDLLAKDCHCI

SEQ ID NO: 49 - protein, 785 aa, Artificial Sequence
  GLP1-GDF15 Fusion Protein 17
HGEGTFTSDVSSYLEEQAAKEFIAWLVKGGGGGGAGGGGAGGGGAGGGGADAHKSEVAHRFKDLGEENFKALVLIAFAQYLQQSPFEDHVKLVNEVTEFAKTCVADESAENCDKSLHTLFGDKLCTVATLRETYGEMADCCAKQEPERNECFLQHKDDNPNLPRLVRPEVDVMCTAFHDNEETFLKKYLYEIARRHPYFYAPELLFFAKRYKAAFTECCQAADKAACLLPKLDELRDEGKASSAKQRLKCASLQKFGERAFKAWAVARLSQRFPKAEFAEVSKLVTDLTKVHTECCHGDLLECADDRADLAKYICENQDSISSKLKECCEKPLLEKSHCIAEVENDEMPADLPSLAADFVESKDVCKNYAEAKDVFLGMFLYEYARRHPDYSVVLLLRLAKTYETTLEKCCAAADPHECYAKVFDEFKPLVEEPQNLIKQNCELFEQLGEYKFQNALLVRYTKKVPQVSTPTLVEVSRNLGKVGSKCCKHPEAKRMPCAEDYLSVVLNQLCVLHEKTPVSDRVTKCCTESLVNRRPCFSALEVDETYVPKEFNAETFTFHADICTLSEKERQIKKQTALVELVKHKPKATKEQLKAVMDDFAAFVEKCCKADDKETCFAEEGKKLVAASQAALGLGAGGGGAGGGGAGGGGAGGGGAGGGGAGGGGAGGGGAGGGGADHCPLGPGRCCRLHTVRASLEDLGWADWVLSPREVQVTMCIGACPSQFRAANMHAQIKTSLHRLKPDTVPAPCCVPASYNPMVLIQKTDTGVSLQTYDDLLAKDCHCI

SEQ ID NO: 50 - protein, 790 aa, Artificial Sequence
  GLP1-GDF15 Fusion Protein 18
HGEGTFTSDVSSYLEEQAAKEFIAWLVKGGGGGGAGGGGAGGGGAGGGGAGGGGADAHKSEVAHRFKDLGEENFKALVLIAFAQYLQQSPFEDHVKLVNEVTEFAKTCVADESAENCDKSLHTLFGDKLCTVATLRETYGEMADCCAKQEPERNECFLQHKDDNPNLPRLVRPEVDVMCTAFHDNEETFLKKYLYEIARRHPYFYAPELLFFAKRYKAAFTECCQAADKAACLLPKLDELRDEGKASSAKQRLKCASLQKFGERAFKAWAVARLSQRFPKAEFAEVSKLVTDLTKVHTECCHGDLLECADDRADLAKYICENQDSISSKLKECCEKPLLEKSHCIAEVENDEMPADLPSLAADFVESKDVCKNYAEAKDVFLGMFLYEYARRHPDYSVVLLLRLAKTYETTLEKCCAAADPHECYAKVFDEFKPLVEEPQNLIKQNCELFEQLGEYKFQNALLVRYTKKVPQVSTPTLVEVSRNLGKVGSKCCKHPEAKRMPCAEDYLSVVLNQLCVLHEKTPVSDRVTKCCTESLVNRRPCFSALEVDETYVPKEFNAETFTFHADICTLSEKERQIKKQTALVELVKHKPKATKEQLKAVMDDFAAFVEKCCKADDKETCFAEEGKKLVAASQAALGLGAGGGGAGGGGAGGGGAGGGGAGGGGAGGGGAGGGGAGGGGADHCPLGPGRCCRLHTVRASLEDLGWADWVLSPREVQVTMCIGACPSQFRAANMHAQIKTSLHRLKPDTVPAPCCVPASYNPMVLIQKTDTGVSLQTYDDLLAKDCHCI

SEQ ID NO: 51 - protein, 807 aa, Artificial Sequence
  GLP1-GDF15 Fusion Protein 19
HGEGTFTSDVSSYLEEQAAKEFIAWLVKGGGAGGGGAGGGGAGGGGAGGGGAGGGGAGGGGAGGGGAGGGGADAHKSEVAHRFKDLGEENFKALVLIAFAQYLQQSPFEDHVKLVNEVTEFAKTCVADESAENCDKSLHTLFGDKLCTVATLRETYGEMADCCAKQEPERNECFLQHKDDNPNLPRLVRPEVDVMCTAFHDNEETFLKKYLYEIARRHPYFYAPELLFFAKRYKAAFTECCQAADKAACLLPKLDELRDEGKASSAKQRLKCASLQKFGERAFKAWAVARLSQRFPKAEFAEVSKLVTDLTKVHTECCHGDLLECADDRADLAKYICENQDSISSKLKECCEKPLLEKSHCIAEVENDEMPADLPSLAADFVESKDVCKNYAEAKDVFLGMFLYEYARRHPDYSVVLLLRLAKTYETTLEKCCAAADPHECYAKVFDEFKPLVEEPQNLIKQNCELFEQLGEYKFQNALLVRYTKKVPQVSTPTLVEVSRNLGKVGSKCCKHPEAKRMPCAEDYLSVVLNQLCVLHEKTPVSDRVTKCCTESLVNRRPCFSALEVDETYVPKEFNAETFTFHADICTLSEKERQIKKQTALVELVKHKPKATKEQLKAVMDDFAAFVEKCCKADDKETCFAEEGKKLVAASQAALGLGSGGGGSGGGGSGGGGSGGGGSGGGGSGGGGSGGGGSGGGGSDHCPLGPGRCCRLHTVRASLEDLGWADWVLSPREVQVTMCIGACPSQFRAANMHAQIKTSLHRLKPDTVPAPCCVPASYNPMVLIQKTDTGVSLQTYDDLLAKDCHCI

SEQ ID NO: 52 - protein, 786 aa, Artificial Sequence
  GLP1-GDF15 Fusion Protein 20
HGEGTFTSDLSKQMEEEAVRLFIEWLKNGGPSSGAPPPSGAGGGGAGGGGADAHKSEVAHRFKDLGEENFKALVLIAFAQYLQQSPFEDHVKLVNEVTEFAKTCVADESAENCDKSLHTLFGDKLCTVATLRETYGEMADCCAKQEPERNECFLQHKDDNPNLPRLVRPEVDVMCTAFHDNEETFLKKYLYEIARRHPYFYAPELLFFAKRYKAAFTECCQAADKAACLLPKLDELRDEGKASSAKQRLKCASLQKFGERAFKAWAVARLSQRFPKAEFAEVSKLVTDLTKVHTECCHGDLLECADDRADLAKYICENQDSISSKLKECCEKPLLEKSHCIAEVENDEMPADLPSLAADFVESKDVCKNYAEAKDVFLGMFLYEYARRHPDYSVVLLLRLAKTYETTLEKCCAAADPHECYAKVFDEFKPLVEEPQNLIKQNCELFEQLGEYKFQNALLVRYTKKVPQVSTPTLVEVSRNLGKVGSKCCKHPEAKRMPCAEDYLSVVLNQLCVLHEKTPVSDRVTKCCTESLVNRRPCFSALEVDETYVPKEFNAETFTFHADICTLSEKERQIKKQTALVELVKHKPKATKEQLKAVMDDFAAFVEKCCKADDKETCFAEEGKKLVAASQAALGLGSGGGGSGGGGSGGGGSGGGGSGGGGSGGGGSGGGGSGGGGSDHCPLGPGRCCRLHTVRASLEDLGWADWVLSPREVQVTMCIGACPSQFRAANMHAQIKTSLHRLKPDTVPAPCCVPASYNPMVLIQKTDTGVSLQTYDDLLAKDCHCI

SEQ ID NO: 53 - protein, 795 aa, Artificial Sequence
  GLP1-GDF15 Fusion Protein 21
HGEGTFTSDVSSYLEEQAAKEFIAWLVKGGGGGGAGGGGAGGGGAGGGGAGGGGAGGGGADAHKSEVAHRFKDLGEENFKALVLIAFAQYLQQSPFEDHVKLVNEVTEFAKTCVADESAENCDKSLHTLFGDKLCTVATLRETYGEMADCCAKQEPERNECFLQHKDDNPNLPRLVRPEVDVMCTAFHDNEETFLKKYLYEIARRHPYFYAPELLFFAKRYKAAFTECCQAADKAACLLPKLDELRDEGKASSAKQRLKCASLQKFGERAFKAWAVARLSQRFPKAEFAEVSKLVTDLTKVHTECCHGDLLECADDRADLAKYICENQDSISSKLKECCEKPLLEKSHCIAEVENDEMPADLPSLAADFVESKDVCKNYAEAKDVFLGMFLYEYARRHPDYSVVLLLRLAKTYETTLEKCCAAADPHECYAKVFDEFKPLVEEPQNLIKQNCELFEQLGEYKFQNALLVRYTKKVPQVSTPTLVEVSRNLGKVGSKCCKHPEAKRMPCAEDYLSVVLNQLCVLHEKTPVSDRVTKCCTESLVNRRPCFSALEVDETYVPKEFNAETFTFHADICTLSEKERQIKKQTALVELVKHKPKATKEQLKAVMDDFAAFVEKCCKADDKETCFAEEGKKLVAASQAALGLGSGGGGSGGGGSGGGGSGGGGSGGGGSGGGGSGGGGSGGGGSDHCPLGPGRCCRLHTVRASLEDLGWADWVLSPREVQVTMCIGACPSQFRAANMHAQIKTSLHRLKPDTVPAPCCVPASYNPMVLIQKTDTGVSLQTYDDLLAKDCHCI

SEQ ID NO: 54 - protein, 790 aa, Artificial Sequence
  GLP1-GDF15 Fusion Protein 22
HGEGTFTSDVSSYLEEQAAKEFIAWLVKGGGGGGAGGGGAGGGGAGGGGAGGGGADAHKSEVAHRFKDLGEENFKALVLIAFAQYLQQSPFEDHVKLVNEVTEFAKTCVADESAENCDKSLHTLFGDKLCTVATLRETYGEMADCCAKQEPERNECFLQHKDDNPNLPRLVRPEVDVMCTAFHDNEETFLKKYLYEIARRHPYFYAPELLFFAKRYKAAFTECCQAADKAACLLPKLDELRDEGKASSAKQRLKCASLQKFGERAFKAWAVARLSQRFPKAEFAEVSKLVTDLTKVHTECCHGDLLECADDRADLAKYICENQDSISSKLKECCEKPLLEKSHCIAEVENDEMPADLPSLAADFVESKDVCKNYAEAKDVFLGMFLYEYARRHPDYSVVLLLRLAKTYETTLEKCCAAADPHECYAKVFDEFKPLVEEPQNLIKQNCELFEQLGEYKFQNALLVRYTKKVPQVSTPTLVEVSRNLGKVGSKCCKHPEAKRMPCAEDYLSVVLNQLCVLHEKTPVSDRVTKCCTESLVNRRPCFSALEVDETYVPKEFNAETFTFHADICTLSEKERQIKKQTALVELVKHKPKATKEQLKAVMDDFAAFVEKCCKADDKETCFAEEGKKLVAASQAALGLGSGGGGSGGGGSGGGGSGGGGSGGGGSGGGGSGGGGSGGGGSDHCPLGPGRCCRLHTVRASLEDLGWADWVLSPREVQVTMCIGACPSQFRAANMHAQIKTSLHRLKPDTVPAPCCVPASYNPMVLIQKTDTGVSLQTYDDLLAKDCHCI

SEQ ID NO: 55 - protein, 795 aa, Artificial Sequence
  GLP1-GDF15 Fusion Protein 23
HGEGTFTSDVSSYLEEQAAKEFIAWLVKGGGGGGSGGGGSGGGGSGGGGSGGGGSGGGGSDAHKSEVAHRFKDLGEENFKALVLIAFAQYLQQSPFEDHVKLVNEVTEFAKTCVADESAENCDKSLHTLFGDKLCTVATLRETYGEMADCCAKQEPERNECFLQHKDDNPNLPRLVRPEVDVMCTAFHDNEETFLKKYLYEIARRHPYFYAPELLFFAKRYKAAFTECCQAADKAACLLPKLDELRDEGKASSAKQRLKCASLQKFGERAFKAWAVARLSQRFPKAEFAEVSKLVTDLTKVHTECCHGDLLECADDRADLAKYICENQDSISSKLKECCEKPLLEKSHCIAEVENDEMPADLPSLAADFVESKDVCKNYAEAKDVFLGMFLYEYARRHPDYSVVLLLRLAKTYETTLEKCCAAADPHECYAKVFDEFKPLVEEPQNLIKQNCELFEQLGEYKFQNALLVRYTKKVPQVSTPTLVEVSRNLGKVGSKCCKHPEAKRMPCAEDYLSVVLNQLCVLHEKTPVSDRVTKCCTESLVNRRPCFSALEVDETYVPKEFNAETFTFHADICTLSEKERQIKKQTALVELVKHKPKATKEQLKAVMDDFAAFVEKCCKADDKETCFAEEGKKLVAASQAALGLGSGGGGSGGGGSGGGGSGGGGSGGGGSGGGGSGGGGSGGGGSDHCPLGPGRCCRLHTVRASLEDLGWADWVLSPREVQVTMCIGACPSQFRAANMHAQIKTSLHRLKPDTVPAPCCVPASYNPMVLIQKTDTGVSLQTYDDLLAKDCHCI

SEQ ID NO: 56 - protein, 790 aa, Artificial Sequence
  GLP1-GDF15 Fusion Protein 24
HGEGTFTSDVSSYLEEQAAKEFIAWLVKGGGGGGSGGGGSGGGGSGGGGSGGGGSDAHKSEVAHRFKDLGEENFKALVLIAFAQYLQQSPFEDHVKLVNEVTEFAKTCVADESAENCDKSLHTLFGDKLCTVATLRETYGEMADCCAKQEPERNECFLQHKDDNPNLPRLVRPEVDVMCTAFHDNEETFLKKYLYEIARRHPYFYAPELLFFAKRYKAAFTECCQAADKAACLLPKLDELRDEGKASSAKQRLKCASLQKFGERAFKAWAVARLSQRFPKAEFAEVSKLVTDLTKVHTECCHGDLLECADDRADLAKYICENQDSISSKLKECCEKPLLEKSHCIAEVENDEMPADLPSLAADFVESKDVCKNYAEAKDVFLGMFLYEYARRHPDYSVVLLLRLAKTYETTLEKCCAAADPHECYAKVFDEFKPLVEEPQNLIKQNCELFEQLGEYKFQNALLVRYTKKVPQVSTPTLVEVSRNLGKVGSKCCKHPEAKRMPCAEDYLSVVLNQLCVLHEKTPVSDRVTKCCTESLVNRRPCFSALEVDETYVPKEFNAETFTFHADICTLSEKERQIKKQTALVELVKHKPKATKEQLKAVMDDFAAFVEKCCKADDKETCFAEEGKKLVAASQAALGLGSGGGGSGGGGSGGGGSGGGGSGGGGSGGGGSGGGGSGGGGSDHCPLGPGRCCRLHTVRASLEDLGWADWVLSPREVQVTMCIGACPSQFRAANMHAQIKTSLHRLKPDTVPAPCCVPASYNPMVLIQKTDTGVSLQTYDDLLAKDCHCI

SEQ ID NO: 57 - protein, 789 aa, Artificial Sequence
  GLP1-GDF15 Fusion Protein 25
HGEGTFTSDVSSYLEEQAAKEFIAWLVKGGASAPAPAPAPAPAPAPAPAPAPGSDAHKSEVAHRFKDLGEENFKALVLIAFAQYLQQSPFEDHVKLVNEVTEFAKTCVADESAENCDKSLHTLFGDKLCTVATLRETYGEMADCCAKQEPERNECFLQHKDDNPNLPRLVRPEVDVMCTAFHDNEETFLKKYLYEIARRHPYFYAPELLFFAKRYKAAFTECCQAADKAACLLPKLDELRDEGKASSAKQRLKCASLQKFGERAFKAWAVARLSQRFPKAEFAEVSKLVTDLTKVHTECCHGDLLECADDRADLAKYICENQDSISSKLKECCEKPLLEKSHCIAEVENDEMPADLPSLAADFVESKDVCKNYAEAKDVFLGMFLYEYARRHPDYSVVLLLRLAKTYETTLEKCCAAADPHECYAKVFDEFKPLVEEPQNLIKQNCELFEQLGEYKFQNALLVRYTKKVPQVSTPTLVEVSRNLGKVGSKCCKHPEAKRMPCAEDYLSVVLNQLCVLHEKTPVSDRVTKCCTESLVNRRPCFSALEVDETYVPKEFNAETFTFHADICTLSEKERQIKKQTALVELVKHKPKATKEQLKAVMDDFAAFVEKCCKADDKETCFAEEGKKLVAASQAALGLGSGGGGSGGGGSGGGGSGGGGSGGGGSGGGGSGGGGSGGGGSDHCPLGPGRCCRLHTVRASLEDLGWADWVLSPREVQVTMCIGACPSQFRAANMHAQIKTSLHRLKPDTVPAPCCVPASYNPMVLIQKTDTGVSLQTYDDLLAKDCHCI

SEQ ID NO: 58 - protein, 807 aa, Artificial Sequence
  GLP1-GDF15 Fusion Protein 26
HGEGTFTSDVSSYLEEQAAKEFIAWLVKGGASGGGGSGGGGSGGGGSGGGGSGGGGSGGGGSGGGGSGGGGSDAHKSEVAHRFKDLGEENFKALVLIAFAQYLQQSPFEDHVKLVNEVTEFAKTCVADESAENCDKSLHTLFGDKLCTVATLRETYGEMADCCAKQEPERNECFLQHKDDNPNLPRLVRPEVDVMCTAFHDNEETFLKKYLYEIARRHPYFYAPELLFFAKRYKAAFTECCQAADKAACLLPKLDELRDEGKASSAKQRLKCASLQKFGERAFKAWAVARLSQRFPKAEFAEVSKLVTDLTKVHTECCHGDLLECADDRADLAKYICENQDSISSKLKECCEKPLLEKSHCIAEVENDEMPADLPSLAADFVESKDVCKNYAEAKDVFLGMFLYEYARRHPDYSVVLLLRLAKTYETTLEKCCAAADPHECYAKVFDEFKPLVEEPQNLIKQNCELFEQLGEYKFQNALLVRYTKKVPQVSTPTLVEVSRNLGKVGSKCCKHPEAKRMPCAEDYLSVVLNQLCVLHEKTPVSDRVTKCCTESLVNRRPCFSALEVDETYVPKEFNAETFTFHADICTLSEKERQIKKQTALVELVKHKPKATKEQLKAVMDDFAAFVEKCCKADDKETCFAEEGKKLVAASQAALGLGSGGGGSGGGGSGGGGSGGGGSGGGGSGGGGSGGGGSGGGGSDHCPLGPGRCCRLHTVRASLEDLGWADWVLSPREVQVTMCIGACPSQFRAANMHAQIKTSLHRLKPDTVPAPCCVPASYNPMVLIQKTDTGVSLQTYDDLLAKDCHCI

SEQ ID NO: 59 - protein, 816 aa, Artificial Sequence
  GLP1-GDF15 Fusion Protein 27
HGEGTFTSDLSKQMEEEAVRLFIEWLKNGGPSSGAPPPSASGGGGSGGGGSGGGGSGGGGSGGGGSGGGGSGGGGSGGGGSDAHKSEVAHRFKDLGEENFKALVLIAFAQYLQQSPFEDHVKLVNEVTEFAKTCVADESAENCDKSLHTLFGDKLCTVATLRETYGEMADCCAKQEPERNECFLQHKDDNPNLPRLVRPEVDVMCTAFHDNEETFLKKYLYEIARRHPYFYAPELLFFAKRYKAAFTECCQAADKAACLLPKLDELRDEGKASSAKQRLKCASLQKFGERAFKAWAVARLSQRFPKAEFAEVSKLVTDLTKVHTECCHGDLLECADDRADLAKYICENQDSISSKLKECCEKPLLEKSHCIAEVENDEMPADLPSLAADFVESKDVCKNYAEAKDVFLGMFLYEYARRHPDYSVVLLLRLAKTYETTLEKCCAAADPHECYAKVFDEFKPLVEEPQNLIKQNCELFEQLGEYKFQNALLVRYTKKVPQVSTPTLVEVSRNLGKVGSKCCKHPEAKRMPCAEDYLSVVLNQLCVLHEKTPVSDRVTKCCTESLVNRRPCFSALEVDETYVPKEFNAETFTFHADICTLSEKERQIKKQTALVELVKHKPKATKEQLKAVMDDFAAFVEKCCKADDKETCFAEEGKKLVAASQAALGLGSGGGGSGGGGSGGGGSGGGGSGGGGSGGGGSGGGGSGGGGSDHCPLGPGRCCRLHTVRASLEDLGWADWVLSPREVQVTMCIGACPSQFRAANMHAQIKTSLHRLKPDTVPAPCCVPASYNPMVLIQKTDTGVSLQTYDDLLAKDCHCI

SEQ ID NO: 60 - protein, 798 aa, Artificial Sequence
  GLP1-GDF15 Fusion Protein 28
HGEGTFTSDLSKQMEEEAVRLFIEWLKNGGPSSGAPPPSASAPAPAPAPAPAPAPAPAPAPGSDAHKSEVAHRFKDLGEENFKALVLIAFAQYLQQSPFEDHVKLVNEVTEFAKTCVADESAENCDKSLHTLFGDKLCTVATLRETYGEMADCCAKQEPERNECFLQHKDDNPNLPRLVRPEVDVMCTAFHDNEETFLKKYLYEIARRHPYFYAPELLFFAKRYKAAFTECCQAADKAACLLPKLDELRDEGKASSAKQRLKCASLQKFGERAFKAWAVARLSQRFPKAEFAEVSKLVTDLTKVHTECCHGDLLECADDRADLAKYICENQDSISSKLKECCEKPLLEKSHCIAEVENDEMPADLPSLAADFVESKDVCKNYAEAKDVFLGMFLYEYARRHPDYSVVLLLRLAKTYETTLEKCCAAADPHECYAKVFDEFKPLVEEPQNLIKQNCELFEQLGEYKFQNALLVRYTKKVPQVSTPTLVEVSRNLGKVGSKCCKHPEAKRMPCAEDYLSVVLNQLCVLHEKTPVSDRVTKCCTESLVNRRPCFSALEVDETYVPKEFNAETFTFHADICTLSEKERQIKKQTALVELVKHKPKATKEQLKAVMDDFAAFVEKCCKADDKETCFAEEGKKLVAASQAALGLGSGGGGSGGGGSGGGGSGGGGSGGGGSGGGGSGGGGSGGGGSDHCPLGPGRCCRLHTVRASLEDLGWADWVLSPREVQVTMCIGACPSQFRAANMHAQIKTSLHRLKPDTVPAPCCVPASYNPMVLIQKTDTGVSLQTYDDLLAKDCHCI

SEQ ID NO: 61 - protein, 789 aa, Artificial Sequence
  GLP1-GDF15 Fusion Protein 29
HSEGTFTSDVSSYLEGQAAKEFIEWLVKGRASAPAPAPAPAPAPAPAPAPAPGSDAHKSEVAHRFKDLGEENFKALVLIAFAQYLQQSPFEDHVKLVNEVTEFAKTCVADESAENCDKSLHTLFGDKLCTVATLRETYGEMADCCAKQEPERNECFLQHKDDNPNLPRLVRPEVDVMCTAFHDNEETFLKKYLYEIARRHPYFYAPELLFFAKRYKAAFTECCQAADKAACLLPKLDELRDEGKASSAKQRLKCASLQKFGERAFKAWAVARLSQRFPKAEFAEVSKLVTDLTKVHTECCHGDLLECADDRADLAKYICENQDSISSKLKECCEKPLLEKSHCIAEVENDEMPADLPSLAADFVESKDVCKNYAEAKDVFLGMFLYEYARRHPDYSVVLLLRLAKTYETTLEKCCAAADPHECYAKVFDEFKPLVEEPQNLIKQNCELFEQLGEYKFQNALLVRYTKKVPQVSTPTLVEVSRNLGKVGSKCCKHPEAKRMPCAEDYLSVVLNQLCVLHEKTPVSDRVTKCCTESLVNRRPCFSALEVDETYVPKEFNAETFTFHADICTLSEKERQIKKQTALVELVKHKPKATKEQLKAVMDDFAAFVEKCCKADDKETCFAEEGKKLVAASQAALGLGSGGGGSGGGGSGGGGSGGGGSGGGGSGGGGSGGGGSGGGGSDHCPLGPGRCCRLHTVRASLEDLGWADWVLSPREVQVTMCIGACPSQFRAANMHAQIKTSLHRLKPDTVPAPCCVPASYNPMVLIQKTDTGVSLQTYDDLLAKDCHCI

SEQ ID NO: 62 - protein, 807 aa, Artificial Sequence
  GLP1-GDF15 Fusion Protein 30
HSEGTFTSDVSSYLEGQAAKEFIEWLVKGRASGGGGSGGGGSGGGGSGGGGSGGGGSGGGGSGGGGSGGGGSDAHKSEVAHRFKDLGEENFKALVLIAFAQYLQQSPFEDHVKLVNEVTEFAKTCVADESAENCDKSLHTLFGDKLCTVATLRETYGEMADCCAKQEPERNECFLQHKDDNPNLPRLVRPEVDVMCTAFHDNEETFLKKYLYEIARRHPYFYAPELLFFAKRYKAAFTECCQAADKAACLLPKLDELRDEGKASSAKQRLKCASLQKFGERAFKAWAVARLSQRFPKAEFAEVSKLVTDLTKVHTECCHGDLLECADDRADLAKYICENQDSISSKLKECCEKPLLEKSHCIAEVENDEMPADLPSLAADFVESKDVCKNYAEAKDVFLGMFLYEYARRHPDYSVVLLLRLAKTYETTLEKCCAAADPHECYAKVFDEFKPLVEEPQNLIKQNCELFEQLGEYKFQNALLVRYTKKVPQVSTPTLVEVSRNLGKVGSKCCKHPEAKRMPCAEDYLSVVLNQLCVLHEKTPVSDRVTKCCTESLVNRRPCFSALEVDETYVPKEFNAETFTFHADICTLSEKERQIKKQTALVELVKHKPKATKEQLKAVMDDFAAFVEKCCKADDKETCFAEEGKKLVAASQAALGLGSGGGGSGGGGSGGGGSGGGGSGGGGSGGGGSGGGGSGGGGSDHCPLGPGRCCRLHTVRASLEDLGWADWVLSPREVQVTMCIGACPSQFRAANMHAQIKTSLHRLKPDTVPAPCCVPASYNPMVLIQKTDTGVSLQTYDDLLAKDCHCI

SEQ ID NO: 63 - protein, 780 aa, Artificial Sequence
  GLP1-GDF15 Fusion Protein 31
HGEGTFTSDVSSYLEEQAAKEFIAWLVKGGGGGGSGGGGSGGGGSDAHKSEVAHRFKDLGEENFKALVLIAFAQYLQQSPFEDHVKLVNEVTEFAKTCVADESAENCDKSLHTLFGDKLCTVATLRETYGEMADCCAKQEPERNECFLQHKDDNPNLPRLVRPEVDVMCTAFHDNEETFLKKYLYEIARRHPYFYAPELLFFAKRYKAAFTECCQAADKAACLLPKLDELRDEGKASSAKQRLKCASLQKFGERAFKAWAVARLSQRFPKAEFAEVSKLVTDLTKVHTECCHGDLLECADDRADLAKYICENQDSISSKLKECCEKPLLEKSHCIAEVENDEMPADLPSLAADFVESKDVCKNYAEAKDVFLGMFLYEYARRHPDYSVVLLLRLAKTYETTLEKCCAAADPHECYAKVFDEFKPLVEEPQNLIKQNCELFEQLGEYKFQNALLVRYTKKVPQVSTPTLVEVSRNLGKVGSKCCKHPEAKRMPCAEDYLSVVLNQLCVLHEKTPVSDRVTKCCTESLVNRRPCFSALEVDETYVPKEFNAETFTFHADICTLSEKERQIKKQTALVELVKHKPKATKEQLKAVMDDFAAFVEKCCKADDKETCFAEEGKKLVAASQAALGLGSGGGGSGGGGSGGGGSGGGGSGGGGSGGGGSGGGGSGGGGSDHCPLGPGRCCRLHTVRASLEDLGWADWVLSPREVQVTMCIGACPSQFRAANMHAQIKTSLHRLKPDTVPAPCCVPASYNPMVLIQKTDTGVSLQTYDDLLAKDCHCI

SEQ ID NO: 64 - protein, 789 aa, Artificial Sequence
  GLP1-GDF15 Fusion Protein 32
HGEGTFTSDLSKQMEEEAVRLFIEWLKNGGPSSGAPPPSGGGGSGGGGSGGGGSDAHKSEVAHRFKDLGEENFKALVLIAFAQYLQQSPFEDHVKLVNEVTEFAKTCVADESAENCDKSLHTLFGDKLCTVATLRETYGEMADCCAKQEPERNECFLQHKDDNPNLPRLVRPEVDVMCTAFHDNEETFLKKYLYEIARRHPYFYAPELLFFAKRYKAAFTECCQAADKAACLLPKLDELRDEGKASSAKQRLKCASLQKFGERAFKAWAVARLSQRFPKAEFAEVSKLVTDLTKVHTECCHGDLLECADDRADLAKYICENQDSISSKLKECCEKPLLEKSHCIAEVENDEMPADLPSLAADFVESKDVCKNYAEAKDVFLGMFLYEYARRHPDYSVVLLLRLAKTYETTLEKCCAAADPHECYAKVFDEFKPLVEEPQNLIKQNCELFEQLGEYKFQNALLVRYTKKVPQVSTPTLVEVSRNLGKVGSKCCKHPEAKRMPCAEDYLSVVLNQLCVLHEKTPVSDRVTKCCTESLVNRRPCFSALEVDETYVPKEFNAETFTFHADICTLSEKERQIKKQTALVELVKHKPKATKEQLKAVMDDFAAFVEKCCKADDKETCFAEEGKKLVAASQAALGLGSGGGGSGGGGSGGGGSGGGGSGGGGSGGGGSGGGGSGGGGSDHCPLGPGRCCRLHTVRASLEDLGWADWVLSPREVQVTMCIGACPSQFRAANMHAQIKTSLHRLKPDTVPAPCCVPASYNPMVLIQKTDTGVSLQTYDDLLAKDCHCI

SEQ ID NO: 65 - protein, 777 aa, Artificial Sequence
  GLP1-GDF15 Fusion Protein 33
HSEGTFTSDVSSYLEGQAAKEFIEWLVKGRASGGGGSGGGGSDAHKSEVAHRFKDLGEENFKALVLIAFAQYLQQSPFEDHVKLVNEVTEFAKTCVADESAENCDKSLHTLFGDKLCTVATLRETYGEMADCCAKQEPERNECFLQHKDDNPNLPRLVRPEVDVMCTAFHDNEETFLKKYLYEIARRHPYFYAPELLFFAKRYKAAFTECCQAADKAACLLPKLDELRDEGKASSAKQRLKCASLQKFGERAFKAWAVARLSQRFPKAEFAEVSKLVTDLTKVHTECCHGDLLECADDRADLAKYICENQDSISSKLKECCEKPLLEKSHCIAEVENDEMPADLPSLAADFVESKDVCKNYAEAKDVFLGMFLYEYARRHPDYSVVLLLRLAKTYETTLEKCCAAADPHECYAKVFDEFKPLVEEPQNLIKQNCELFEQLGEYKFQNALLVRYTKKVPQVSTPTLVEVSRNLGKVGSKCCKHPEAKRMPCAEDYLSVVLNQLCVLHEKTPVSDRVTKCCTESLVNRRPCFSALEVDETYVPKEFNAETFTFHADICTLSEKERQIKKQTALVELVKHKPKATKEQLKAVMDDFAAFVEKCCKADDKETCFAEEGKKLVAASQAALGLGSGGGGSGGGGSGGGGSGGGGSGGGGSGGGGSGGGGSGGGGSDHCPLGPGRCCRLHTVRASLEDLGWADWVLSPREVQVTMCIGACPSQFRAANMHAQIKTSLHRLKPDTVPAPCCVPASYNPMVLIQKTDTGVSLQTYDDLLAKDCHCI

SEQ ID NO: 66 - protein, 779 aa, Artificial Sequence
  GLP1-GDF15 Fusion Protein 34
HSEGTFTSDVSSYLEGQAAKEFIEWLVKGRASAPAPAPAPAPGSDAHKSEVAHRFKDLGEENFKALVLIAFAQYLQQSPFEDHVKLVNEVTEFAKTCVADESAENCDKSLHTLFGDKLCTVATLRETYGEMADCCAKQEPERNECFLQHKDDNPNLPRLVRPEVDVMCTAFHDNEETFLKKYLYEIARRHPYFYAPELLFFAKRYKAAFTECCQAADKAACLLPKLDELRDEGKASSAKQRLKCASLQKFGERAFKAWAVARLSQRFPKAEFAEVSKLVTDLTKVHTECCHGDLLECADDRADLAKYICENQDSISSKLKECCEKPLLEKSHCIAEVENDEMPADLPSLAADFVESKDVCKNYAEAKDVFLGMFLYEYARRHPDYSVVLLLRLAKTYETTLEKCCAAADPHECYAKVFDEFKPLVEEPQNLIKQNCELFEQLGEYKFQNALLVRYTKKVPQVSTPTLVEVSRNLGKVGSKCCKHPEAKRMPCAEDYLSVVLNQLCVLHEKTPVSDRVTKCCTESLVNRRPCFSALEVDETYVPKEFNAETFTFHADICTLSEKERQIKKQTALVELVKHKPKATKEQLKAVMDDFAAFVEKCCKADDKETCFAEEGKKLVAASQAALGLGSGGGGSGGGGSGGGGSGGGGSGGGGSGGGGSGGGGSGGGGSDHCPLGPGRCCRLHTVRASLEDLGWADWVLSPREVQVTMCIGACPSQFRAANMHAQIKTSLHRLKPDTVPAPCCVPASYNPMVLIQKTDTGVSLQTYDDLLAKDCHCI

SEQ ID NO: 67 - protein, 786 aa, Artificial Sequence
  GLP1-GDF15 Fusion Protein 35
HGEGTFTSDLSKQMEEEAVRLFIEWLKNGGPSSGAPPPSASGGGGSGGGGSDAHKSEVAHRFKDLGEENFKALVLIAFAQYLQQSPFEDHVKLVNEVTEFAKTCVADESAENCDKSLHTLFGDKLCTVATLRETYGEMADCCAKQEPERNECFLQHKDDNPNLPRLVRPEVDVMCTAFHDNEETFLKKYLYEIARRHPYFYAPELLFFAKRYKAAFTECCQAADKAACLLPKLDELRDEGKASSAKQRLKCASLQKFGERAFKAWAVARLSQRFPKAEFAEVSKLVTDLTKVHTECCHGDLLECADDRADLAKYICENQDSISSKLKECCEKPLLEKSHCIAEVENDEMPADLPSLAADFVESKDVCKNYAEAKDVFLGMFLYEYARRHPDYSVVLLLRLAKTYETTLEKCCAAADPHECYAKVFDEFKPLVEEPQNLIKQNCELFEQLGEYKFQNALLVRYTKKVPQVSTPTLVEVSRNLGKVGSKCCKHPEAKRMPCAEDYLSVVLNQLCVLHEKTPVSDRVTKCCTESLVNRRPCFSALEVDETYVPKEFNAETFTFHADICTLSEKERQIKKQTALVELVKHKPKATKEQLKAVMDDFAAFVEKCCKADDKETCFAEEGKKLVAASQAALGLGSGGGGSGGGGSGGGGSGGGGSGGGGSGGGGSGGGGSGGGGSDHCPLGPGRCCRLHTVRASLEDLGWADWVLSPREVQVTMCIGACPSQFRAANMHAQIKTSLHRLKPDTVPAPCCVPASYNPMVLIQKTDTGVSLQTYDDLLAKDCHCI

SEQ ID NO: 68 - protein, 788 aa, Artificial Sequence
  GLP1-GDF15 Fusion Protein 36
HGEGTFTSDLSKQMEEEAVRLFIEWLKNGGPSSGAPPPSASAPAPAPAPAPGSDAHKSEVAHRFKDLGEENFKALVLIAFAQYLQQSPFEDHVKLVNEVTEFAKTCVADESAENCDKSLHTLFGDKLCTVATLRETYGEMADCCAKQEPERNECFLQHKDDNPNLPRLVRPEVDVMCTAFHDNEETFLKKYLYEIARRHPYFYAPELLFFAKRYKAAFTECCQAADKAACLLPKLDELRDEGKASSAKQRLKCASLQKFGERAFKAWAVARLSQRFPKAEFAEVSKLVTDLTKVHTECCHGDLLECADDRADLAKYICENQDSISSKLKECCEKPLLEKSHCIAEVENDEMPADLPSLAADFVESKDVCKNYAEAKDVFLGMFLYEYARRHPDYSVVLLLRLAKTYETTLEKCCAAADPHECYAKVFDEFKPLVEEPQNLIKQNCELFEQLGEYKFQNALLVRYTKKVPQVSTPTLVEVSRNLGKVGSKCCKHPEAKRMPCAEDYLSVVLNQLCVLHEKTPVSDRVTKCCTESLVNRRPCFSALEVDETYVPKEFNAETFTFHADICTLSEKERQIKKQTALVELVKHKPKATKEQLKAVMDDFAAFVEKCCKADDKETCFAEEGKKLVAASQAALGLGSGGGGSGGGGSGGGGSGGGGSGGGGSGGGGSGGGGSGGGGSDHCPLGPGRCCRLHTVRASLEDLGWADWVLSPREVQVTMCIGACPSQFRAANMHAQIKTSLHRLKPDTVPAPCCVPASYNPMVLIQKTDTGVSLQTYDDLLAKDCHCI

SEQ ID NO: 69 - protein, 777 aa, Artificial Sequence
  GLP1-GDF15 Fusion Protein 37
HGEGTFTSDVSSYLEEQAAKEFIAWLVKGGASGGGGSGGGGSDAHKSEVAHRFKDLGEENFKALVLIAFAQYLQQSPFEDHVKLVNEVTEFAKTCVADESAENCDKSLHTLFGDKLCTVATLRETYGEMADCCAKQEPERNECFLQHKDDNPNLPRLVRPEVDVMCTAFHDNEETFLKKYLYEIARRHPYFYAPELLFFAKRYKAAFTECCQAADKAACLLPKLDELRDEGKASSAKQRLKCASLQKFGERAFKAWAVARLSQRFPKAEFAEVSKLVTDLTKVHTECCHGDLLECADDRADLAKYICENQDSISSKLKECCEKPLLEKSHCIAEVENDEMPADLPSLAADFVESKDVCKNYAEAKDVFLGMFLYEYARRHPDYSVVLLLRLAKTYETTLEKCCAAADPHECYAKVFDEFKPLVEEPQNLIKQNCELFEQLGEYKFQNALLVRYTKKVPQVSTPTLVEVSRNLGKVGSKCCKHPEAKRMPCAEDYLSVVLNQLCVLHEKTPVSDRVTKCCTESLVNRRPCFSALEVDETYVPKEFNAETFTFHADICTLSEKERQIKKQTALVELVKHKPKATKEQLKAVMDDFAAFVEKCCKADDKETCFAEEGKKLVAASQAALGLGSGGGGSGGGGSGGGGSGGGGSGGGGSGGGGSGGGGSGGGGSDHCPLGPGRCCRLHTVRASLEDLGWADWVLSPREVQVTMCIGACPSQFRAANMHAQIKTSLHRLKPDTVPAPCCVPASYNPMVLIQKTDTGVSLQTYDDLLAKDCHCI

SEQ ID NO: 70 - protein, 779 aa, Artificial Sequence
  GLP1-GDF15 Fusion Protein 38
HGEGTFTSDVSSYLEEQAAKEFIAWLVKGGASAPAPAPAPAPGSDAHKSEVAHRFKDLGEENFKALVLIAFAQYLQQSPFEDHVKLVNEVTEFAKTCVADESAENCDKSLHTLFGDKLCTVATLRETYGEMADCCAKQEPERNECFLQHKDDNPNLPRLVRPEVDVMCTAFHDNEETFLKKYLYEIARRHPYFYAPELLFFAKRYKAAFTECCQAADKAACLLPKLDELRDEGKASSAKQRLKCASLQKFGERAFKAWAVARLSQRFPKAEFAEVSKLVTDLTKVHTECCHGDLLECADDRADLAKYICENQDSISSKLKECCEKPLLEKSHCIAEVENDEMPADLPSLAADFVESKDVCKNYAEAKDVFLGMFLYEYARRHPDYSVVLLLRLAKTYETTLEKCCAAADPHECYAKVFDEFKPLVEEPQNLIKQNCELFEQLGEYKFQNALLVRYTKKVPQVSTPTLVEVSRNLGKVGSKCCKHPEAKRMPCAEDYLSVVLNQLCVLHEKTPVSDRVTKCCTESLVNRRPCFSALEVDETYVPKEFNAETFTFHADICTLSEKERQIKKQTALVELVKHKPKATKEQLKAVMDDFAAFVEKCCKADDKETCFAEEGKKLVAASQAALGLGSGGGGSGGGGSGGGGSGGGGSGGGGSGGGGSGGGGSGGGGSDHCPLGPGRCCRLHTVRASLEDLGWADWVLSPREVQVTMCIGACPSQFRAANMHAQIKTSLHRLKPDTVPAPCCVPASYNPMVLIQKTDTGVSLQTYDDLLAKDCHCI

SEQ ID NO: 71 - protein, 780 aa, Artificial Sequence
  GLP1-GDF15 Fusion Protein 39
HSEGTFTSDVSSYLEGQAAKEFIEWLVKGRGGGGSGGGGSGGGGSDAHKSEVAHRFKDLGEENFKALVLIAFAQYLQQSPFEDHVKLVNEVTEFAKTCVADESAENCDKSLHTLFGDKLCTVATLRETYGEMADCCAKQEPERNECFLQHKDDNPNLPRLVRPEVDVMCTAFHDNEETFLKKYLYEIARRHPYFYAPELLFFAKRYKAAFTECCQAADKAACLLPKLDELRDEGKASSAKQRLKCASLQKFGERAFKAWAVARLSQRFPKAEFAEVSKLVTDLTKVHTECCHGDLLECADDRADLAKYICENQDSISSKLKECCEKPLLEKSHCIAEVENDEMPADLPSLAADFVESKDVCKNYAEAKDVFLGMFLYEYARRHPDYSVVLLLRLAKTYETTLEKCCAAADPHECYAKVFDEFKPLVEEPQNLIKQNCELFEQLGEYKFQNALLVRYTKKVPQVSTPTLVEVSRNLGKVGSKCCKHPEAKRMPCAEDYLSVVLNQLCVLHEKTPVSDRVTKCCTESLVNRRPCFSALEVDETYVPKEFNAETFTFHADICTLSEKERQIKKQTALVELVKHKPKATKEQLKAVMDDFAAFVEKCCKADDKETCFAEEGKKLVAASQAALGLGSGGGGSGGGGSGGGGSGGGGSGGGGSGGGGSGGGGSGGGGSDHCPLGPGRCCRLHTVRASLEDLGWADWVLSPREVQVTMCIGACPSQFRAANMHAQIKTSLHRLKPDTVPAPCCVPASYNPMVLIQKTDTGVSLQTYDDLLAKDCHCI

SEQ ID NO: 72 - protein, 780 aa, Artificial Sequence
  GLP1-GDF15 Fusion Protein 40
HGEGTFTSDVSSYLEEQAAKEFIAWLVKGGGGGGSGGGGSGGGGSDAHKSEVAHRFKDLGEETFKALVLVAFAQYLQQSPFEDHVKLVNEVTEFAKTCVADESAENCDKSLHTLFGDKLCTVATLRETYGEMADCCAKQEPERNECFLQHKDDNPNLPRLVRPEVDVMCTAFHDNEETFLKKYLYEIARRHPYFYAPELLFFAARYKAAFTECCQAADKAACLLPKLDELRDEGKASSAKQRLKCASLQKFGERAFKAWAVARLSQRFPKAEFAEVSKLVTDLTKVHTECCHGDLLECADDRADLAKYICENQDSISSKLKECCEKPLLEKSHCLAEVENDEMPADLPSLAADFVESKDVCKNYAEAKDVFLGMFLYEYARRHPDYSVVLLLRLAKTYETTLEKCCAAADPHECYAKVFDEFKPLVEEPQNLIKQNCELFEQLGEYKFQNALLVRYTKKVPQVSTPTLVEVSRNLGKVGSKCCKHPEAKRMPCAEDYLSVVLNQLCVLHEKTPVSDRVTKCCTESLVNRRPCFSALEVDETYVPKEFNAETFTFHADICTLSEKERQIKKQTALAELVKHKPKATKEQLKTVMDDFAAFVEKCCKADDKETCFAEEGKKLVAASQAALGLGSGGGGSGGGGSGGGGSGGGGSGGGGSGGGGSGGGGSGGGGSDHCPLGPGRCCRLHTVRASLEDLGWADWVLSPREVQVTMCIGACPSQFRAANMHAQIKTSLHRLKPDTVPAPCCVPASYNPMVLIQKTDTGVSLQTYDDLLAKDCHCI

SEQ ID NO: 73 - protein, 780 aa, Artificial Sequence
  GLP1-GDF15 Fusion Protein 41
HGEGTFTSDVSSYLEEQAAKEFIAWLVKGGGGGGSGGGGSGGGGSDAHKSEVAHRFKDLGEETFKALVLVAFAQYLQQSPFEDHVKLVNEVTEFAKTCVADESAENCDKSLHTLFGDKLCTVATLRETYGEMADCCAKQEPERNECFLQHKDDNPNLPRLVRPEVDVMCTAFHDNEETFLKKYLYEIARRHPYFYAPELLFFAARYKAAFTECCQAADKAACLLPKLDELRDEGKASSAKQRLKCASLQKFGERAFKAWAVARLSQRFPKAEFAEVSKLVTDLTKVHTECCHGDLLECADDRADLAKYICENQDSISSKLKECCEKPLLEKSHCLAEVENDEMPADLPSLAADFVESKDVCKNYAEAKDVFLGMFLYEYARRHPDYSVVLLLRLAKTYETTLEKCCAAADPHECYAKVFDEFKPLVEEPQNLIKQNCELFEQLGEYKFQNALLVRYTKKVPQVSTPTLVEVSRNLGKVGSKCCKHPEAKRMPCAEDYLSVVLNQLCVLHEKTPVSDRVTKCCTESLVNRRPCFSALEVDETYVPKEFNAETFTFHADICTLSEKERQIKKQTALAELVKHKPKATKEQLKTVMDDFAAFVEKCCKADDKETCFAEEGKKLVAASQAALGLGSGGGGSGGGGSGGGGSGGGGSGGGGSGGGGSGGGGSGGGGSDHCPLGPGRCCRLHTVRASLEDLGWADWVLSPREVQVTMCIGACPSQFRAANMHAQIKTSLHRLKPDTVPAPCCVPASYNPMVLRQKTDTGVSLQTYDDLLAKDCHCI

SEQ ID NO: 74 - protein, 778 aa, Artificial Sequence
  GLP1-GDF15 Fusion Protein 42
EGTFTSDVSSYLEEQAAKEFIAWLVKGGGGGGSGGGGSGGGGSDAHKSEVAHRFKDLGEETFKALVLVAFAQYLQQSPFEDHVKLVNEVTEFAKTCVADESAENCDKSLHTLFGDKLCTVATLRETYGEMADCCAKQEPERNECFLQHKDDNPNLPRLVRPEVDVMCTAFHDNEETFLKKYLYEIARRHPYFYAPELLFFAARYKAAFTECCQAADKAACLLPKLDELRDEGKASSAKQRLKCASLQKFGERAFKAWAVARLSQRFPKAEFAEVSKLVTDLTKVHTECCHGDLLECADDRADLAKYICENQDSISSKLKECCEKPLLEKSHCLAEVENDEMPADLPSLAADFVESKDVCKNYAEAKDVFLGMFLYEYARRHPDYSVVLLLRLAKTYETTLEKCCAAADPHECYAKVFDEFKPLVEEPQNLIKQNCELFEQLGEYKFQNALLVRYTKKVPQVSTPTLVEVSRNLGKVGSKCCKHPEAKRMPCAEDYLSVVLNQLCVLHEKTPVSDRVTKCCTESLVNRRPCFSALEVDETYVPKEFNAETFTFHADICTLSEKERQIKKQTALAELVKHKPKATKEQLKTVMDDFAAFVEKCCKADDKETCFAEEGKKLVAASQAALGLGSGGGGSGGGGSGGGGSGGGGSGGGGSGGGGSGGGGSGGGGSDHCPLGPGRCCRLHTVRASLEDLGWADWVLSPREVQVTMCIGACPSQFRAANMHAQIKTSLHRLKPDTVPAPCCVPASYNPMVLIQKTDTGVSLQTYDDLLAKDCHCI

SEQ ID NO: 75 - protein, 735 aa, Artificial Sequence
  GSA-GDF15 fusion protein
DAHKSEVAHRFKDLGEETFKALVLVAFAQYLQQSPFEDHVKLVNEVTEFAKTCVADESAENCDKSLHTLFGDKLCTVATLRETYGEMADCCAKQEPERNECFLQHKDDNPNLPRLVRPEVDVMCTAFHDNEETFLKKYLYEIARRHPYFYAPELLFFAARYKAAFTECCQAADKAACLLPKLDELRDEGKASSAKQRLKCASLQKFGERAFKAWAVARLSQRFPKAEFAEVSKLVTDLTKVHTECCHGDLLECADDRADLAKYICENQDSISSKLKECCEKPLLEKSHCLAEVENDEMPADLPSLAADFVESKDVCKNYAEAKDVFLGMFLYEYARRHPDYSVVLLLRLAKTYETTLEKCCAAADPHECYAKVFDEFKPLVEEPQNLIKQNCELFEQLGEYKFQNALLVRYTKKVPQVSTPTLVEVSRNLGKVGSKCCKHPEAKRMPCAEDYLSVVLNQLCVLHEKTPVSDRVTKCCTESLVNRRPCFSALEVDETYVPKEFNAETFTFHADICTLSEKERQIKKQTALAELVKHKPKATKEQLKTVMDDFAAFVEKCCKADDKETCFAEEGKKLVAASQAALGLGSGGGGSGGGGSGGGGSGGGGSGGGGSGGGGSGGGGSGGGGSDHCPLGPGRCCRLHTVRASLEDLGWADWVLSPREVQVTMCIGACPSQFRAANMHAQIKTSLHRLKPDTVPAPCCVPASYNPMVLIQKTDTGVSLQTYDDLLAKDCHCI

SEQ ID NO: 76 - protein, 20 aa, Artificial Sequence
  HSE peptide
HSEGTFTSDVSSYLEGQAAK

SEQ ID NO: 77 - protein, 20 aa, Artificial Sequence
  HGE-1 peptide
HGEGTFTSDVSSYLEEQAAK

SEQ ID NO: 78 - protein, 12 aa, Artificial Sequence
  HGE-2 peptide
HGEGTFTSDLSK

SEQ ID NO: 79 - protein, 21 aa, Artificial Sequence
  ALV peptide
ALVLIAFAQYLQQSPFEDHVK

SEQ ID NO: 80 - protein, 16 aa, Artificial Sequence
  TDT peptide
TDTGVSLQTYDDLLAK

SEQ ID NO: 81 - protein, 727 aa, Artificial Sequence
  HSA-GDF15 fusion protein
EFHHHHHHDAHKSEVAHRFKDLGEENFKALVLIAFAQYLQQSPFEDHVKLVNEVTEFAKTCVADESAENCDKSLHTLFGDKLCTVATLRETYGEMADCCAKQEPERNECFLQHKDDNPNLPRLVRPEVDVMCTAFHDNEETFLKKYLYEIARRHPYFYAPELLFFAKRYKAAFTECCQAADKAACLLPKLDELRDEGKASSAKQRLKCASLQKFGERAFKAWAVARLSQRFPKAEFAEVSKLVTDLTKVHTECCHGDLLECADDRADLAKYICENQDSISSKLKECCEKPLLEKSHCIAEVENDEMPADLPSLAADFVESKDVCKNYAEAKDVFLGMFLYEYARRHPDYSVVLLLRLAKTYETTLEKCCAAADPHECYAKVFDEFKPLVEEPQNLIKQNCELFEQLGEYKFQNALLVRYTKKVPQVSTPTLVEVSRNLGKVGSKCCKHPEAKRMPCAEDYLSVVLNQLCVLHEKTPVSDRVTKCCTESLVNRRPCFSALEVDETYVPKEFNAETFTFHADICTLSEKERQIKKQTALVELVKHKPKATKEQLKAVMDDFAAFVEKCCKADDKETCFAEEGKKLVAASQAALGLGSGGGGSGGGGSGGGGSGGGGSARNGDHCPLGPGRCCRLHTVRASLEDLGWADWVLSPREVQVTMCIGACPSQFRAANMHAQIKTSLHRLKPDTVPAPCCVPASYNPMVLIQKTDTGVSLQTYDDLLAKDCHCI

SEQ ID NO: 82 - protein, 16 aa, Artificial Sequence
  VVS peptide
VVSVLTVLHQDWLNGK

SEQ ID NO: 83 - protein, 713 aa, Artificial Sequence
  HSA-GDF15 fusion peptide
DAHKSEVAHRFKDLGEENFKALVLIAFAQYLQQSPFEDHVKLVNEVTEFAKTCVADESAENCDKSLHTLFGDKLCTVATLRETYGEMADCCAKQEPERNECFLQHKDDNPNLPRLVRPEVDVMCTAFHDNEETFLKKYLYEIARRHPYFYAPELLFFAKRYKAAFTECCQAADKAACLLPKLDELRDEGKASSAKQRLKCASLQKFGERAFKAWAVARLSQRFPKAEFAEVSKLVTDLTKVHTECCHGDLLECADDRADLAKYICENQDSISSKLKECCEKPLLEKSHCIAEVENDEMPADLPSLAADFVESKDVCKNYAEAKDVFLGMFLYEYARRHPDYSVVLLLRLAKTYETTLEKCCAAADPHECYAKVFDEFKPLVEEPQNLIKQNCELFEQLGEYKFQNALLVRYTKKVPQVSTPTLVEVSRNLGKVGSKCCKHPEAKRMPCAEDYLSVVLNQLCVLHEKTPVSDRVTKCCTESLVNRRPCFSALEVDETYVPKEFNAETFTFHADICTLSEKERQIKKQTALVELVKHKPKATKEQLKAVMDDFAAFVEKCCKADDKETCFAEEGKKLVAASQAALGLAPAPAPAPAPAPAPAPAPAPDHCPLGPGRCCRLHTVRASLEDLGWADWVLSPREVQVTMCIGACPSQFRAANMHAQIKTSLHRLKPDTVPAPCCVPASYNPMVLIQKTDTGVSLQTYDDLLAKDCHCI

SEQ ID NO: 84 - protein, 762 aa, Artificial Sequence
  GLP1-GDF15 (I89R) fusion peptide
HGEGTFTSDLSKQMEEEAVRLFIEWLKNGGPSSGAPPPSAPAPAPAPAPDAHKSEVAHRFKDLGEENFKALVLIAFAQYLQQSPFEDHVKLVNEVTEFAKTCVADESAENCDKSLHTLFGDKLCTVATLRETYGEMADCCAKQEPERNECFLQHKDDNPNLPRLVRPEVDVMCTAFHDNEETFLKKYLYEIARRHPYFYAPELLFFAKRYKAAFTECCQAADKAACLLPKLDELRDEGKASSAKQRLKCASLQKFGERAFKAWAVARLSQRFPKAEFAEVSKLVTDLTKVHTECCHGDLLECADDRADLAKYICENQDSISSKLKECCEKPLLEKSHCIAEVENDEMPADLPSLAADFVESKDVCKNYAEAKDVFLGMFLYEYARRHPDYSVVLLLRLAKTYETTLEKCCAAADPHECYAKVFDEFKPLVEEPQNLIKQNCELFEQLGEYKFQNALLVRYTKKVPQVSTPTLVEVSRNLGKVGSKCCKHPEAKRMPCAEDYLSVVLNQLCVLHEKTPVSDRVTKCCTESLVNRRPCFSALEVDETYVPKEFNAETFTFHADICTLSEKERQIKKQTALVELVKHKPKATKEQLKAVMDDFAAFVEKCCKADDKETCFAEEGKKLVAASQAALGLAPAPAPAPAPAPAPAPAPAPDHCPLGPGRCCRLHTVRASLEDLGWADWVLSPREVQVTMCIGACPSQFRAANMHAQIKTSLHRLKPDTVPAPCCVPASYNPMVLRQKTDTGVSLQTYDDLLAKDCHCI